European Patent Application EP 4 083 068 A9, published July 19, 2023. Title: ANTI-NGF ANTIBODY AND ANTIGEN-BINDING FRAGMENT THEREOF,PREPARATION METHOD THEREROFR, AND APPLICATION THEREOF. Applicant: XIYUAN ANJIAN MEDCINE (SHANGHAI) CO., LTD. Application EP21852225.8. The sequence listing filed with the application follows.

SEQUENCE LISTING (64 sequences)

SEQ ID NO: 1 - protein, 123 aa, Artificial Sequence
  VH CDR
QVQLQQSGAELVRPGASVTLSCKASGYTFTDYEMHWVRQTPVHGLEWIGAIDPETGGTAYNQKFKGKATLTADKSSSTAYMELRSLTSEDSAVYYCRRGANLNHYGNDEGSYWGQGTLVTVSA

SEQ ID NO: 2 - DNA, 369 bp, Artificial Sequence
  Polynucleotide
caggttcaactgcagcagtctggggctgagctggtgaggcctggggcttcagtgacgctgtcctgcaaggcttcgggctacacatttactgactatgaaatgcactgggtgaggcagacacctgtgcatggcctggaatggattggagctattgatcctgaaactggtggtactgcctacaatcagaagttcaagggcaaggccacactgactgcagacaaatcctccagcacagcctacatggagctccgcagcctgacatctgaggactctgccgtctattactgtagaagaggggcaaatcttaatcactatggtaacgacgagggttcttactggggccaagggactctggtcactgtctctgca

SEQ ID NO: 3 - protein, 112 aa, Artificial Sequence
  VL CDR
DVVMTQTPLTLSVTIGQPASISCKSSQSLLHSVGKTYLNWLLQRPGQSPKRLIYLVSKLDSGVPDRFTGSGSGTDFTLKISRVEAEDLGVYFCWQGTHLPQTFGGGTKLEIK

SEQ ID NO: 4 - DNA, 336 bp, Artificial Sequence
  Polynucleotide
gatgttgtgatgacccagactccactcactttgtcggttaccattggacaaccagcctccatctcttgtaagtcaagtcagagcctcttacatagtgttggaaagacatatttgaattggttgttacagaggccaggccagtctccaaagcgcctaatctatctggtgtctaaactggactctggagtccctgacaggttcactggcagtggatcagggacagatttcacactgaaaatcagcagagtggaggctgaggatttgggagtttatttttgctggcaaggtacacatcttcctcagacgttcggtggaggcaccaagctggaaatcaaa

SEQ ID NO: 5 - protein, 119 aa, Artificial Sequence
  VH CDR
QVQLKESGPGLVAPSQSLSITCTVSGFSLTGYAVNWVRQPPGKGLEWLGMIWFDGSTDYNSALKSRLSISKDNSKSQVFLKMNSLQTDDTARYYCARDYYGSSWYFDVWGAGTTVTVSS

SEQ ID NO: 6 - DNA, 357 bp, Artificial Sequence
  Polynucleotide
caggtgcagctgaaggagtcaggacctggcctggtggcgccctcacagagcctgtccatcacatgcaccgtctcagggttctcattaaccggctatgctgtaaactgggttcgccagcctccaggaaagggtctggagtggctgggaatgatatggtttgatggaagcacagactataattcagctctcaaatccagactgagcatcagcaaggacaactccaagagccaagttttcttaaaaatgaacagtctgcaaactgatgacacagccaggtactactgtgccagagactactacggtagtagctggtacttcgatgtctggggcgcagggaccacggtcaccgtctcctca

SEQ ID NO: 7 - protein, 107 aa, Artificial Sequence
  VL CDR
DIQMTQTTSSLSASLGDRVTISCRASQDISYYLNWYQQKPDGTVKLLIYYTSRLHSGVPSRFSGSGSGTDYSLTISNLEQEDIATYFCQQGNTLPRTFGGGTKLDIK

SEQ ID NO: 8 - DNA, 321 bp, Artificial Sequence
  Polynucleotide
gatatccagatgacacagactacatcctccctgtctgcctctctgggagacagagtcaccatcagttgcagggcaagtcaggacattagctattatttaaactggtatcagcagaaaccagatggaactgttaaactcctgatctactacacatcaagattacactcaggagtcccatcaaggttcagtggcagtgggtctggaacagattattctctcaccattagcaacctggagcaagaagatattgccacttacttttgccaacagggtaatacgcttcctcggacgttcggtggaggcaccaagctggacatcaaa

SEQ ID NO: 9 - protein, 121 aa, Artificial Sequence
  VH CDR
QVQLKESGPGLVAPSQSLSITCTVSGFSLTGYGVNWVRQPPGKGLEWLGMIWFDGSTDYNSALKSRLSISKDNSKSQVFLKMNSLQTDDTARYYCAREGYYYGTTYYFDYWGQGTTLTVSS

SEQ ID NO: 10 - DNA, 363 bp, Artificial Sequence
  Polynucleotide
caggtgcagctgaaggagtcaggacctggcctggtggcgccctcacagagcctgtccatcacatgcaccgtctcagggttctcattaaccggctatggtgtaaactgggttcgccagcctccaggaaagggtctggagtggctgggaatgatatggtttgatggaagcacagactataattcagctctcaaatccagactgagcatcagcaaggacaactccaagagccaagttttcttaaaaatgaacagtctgcaaactgatgacacagccaggtactactgtgccagagagggttattactacggtactacctactactttgactactggggccaaggcaccactctcacagtctcctca

SEQ ID NO: 11 - protein, 107 aa, Artificial Sequence
  VL CDR
DIQMTQTTSSLSASLGDRVTISCRASQDISNYLNWYQQKPDGTVKLLIYYTSRLHSGVPSRFSGSGSGTDYSLTISNLEQEDIATYFCQQGNTLPRTFGGGTKLEIK

SEQ ID NO: 12 - DNA, 321 bp, Artificial Sequence
  Polynucleotide
gatatccagatgacacagactacatcctccctgtctgcctctctgggagacagagtcaccatcagttgcagggcaagtcaggacattagcaattatttaaactggtatcagcagaaaccagatggaactgttaaactcctgatctactacacatcaagattacactcaggagtcccatcaaggttcagtggcagtgggtctggaacagattattctctcaccattagcaacctggagcaagaagatattgccacttacttttgccaacagggtaatacgcttcctcggacgttcggtggaggcaccaagctggaaatcaaa

SEQ ID NO: 13 - protein, 10 aa, Artificial Sequence
  43E5 CDR-H1
GYTFTDYEMH

SEQ ID NO: 14 - protein, 17 aa, Artificial Sequence
  43E5 CDR-H2
AIDPETGGTAYNQKFKG

SEQ ID NO: 15 - protein, 16 aa, Artificial Sequence
  43E5 CDR-H3
RRGANLNHYGNDEGSY

SEQ ID NO: 16 - protein, 10 aa, Artificial Sequence
  137H8 CDR-H1
GFSLTGYAVN

SEQ ID NO: 17 - protein, 16 aa, Artificial Sequence
  137H8 CDR-H2
MIWFDGSTDYNSALKS

SEQ ID NO: 18 - protein, 13 aa, Artificial Sequence
  137H8 CDR-H3
ARDYYGSSWYFDV

SEQ ID NO: 19 - protein, 10 aa, Artificial Sequence
  138E12 CDR-H1
GFSLTGYGVN

SEQ ID NO: 20 - protein, 16 aa, Artificial Sequence
  138E12 CDR-H2
MIWFDGSTDYNSALKS

SEQ ID NO: 21 - protein, 15 aa, Artificial Sequence
  138E12 CDR-H3
AREGYYYGTTYYFDY

SEQ ID NO: 22 - protein, 16 aa, Artificial Sequence
  43E5 CDR-L1
KSSQSLLHSVGKTYLN

SEQ ID NO: 23 - protein, 7 aa, Artificial Sequence
  43E5 CDR-L2
LVSKLDS

SEQ ID NO: 24 - protein, 9 aa, Artificial Sequence
  43E5 CDR-L3
WQGTHLPQT

SEQ ID NO: 25 - protein, 11 aa, Artificial Sequence
  137H8 CDR-L1
RASQDISYYLN

SEQ ID NO: 26 - protein, 7 aa, Artificial Sequence
  137H8 CDR-L2
YTSRLHS

SEQ ID NO: 27 - protein, 9 aa, Artificial Sequence
  137H8 CDR-L3
QQGNTLPRT

SEQ ID NO: 28 - protein, 11 aa, Artificial Sequence
  138E12 CDR-L1
RASQDISNYLN

SEQ ID NO: 29 - protein, 7 aa, Artificial Sequence
  138E12 CDR-L2
YTSRLHS

SEQ ID NO: 30 - protein, 9 aa, Artificial Sequence
  138E12 CDR-L3
QQGNTLPRT

SEQ ID NO: 31 - protein, 112 aa, Artificial Sequence
  Amino acid sequence of light chain
DVVMTQSPLSLPVTLGQPASISCKSSQSLLHSVGKTYLNWLQQRPGQSPRRLIYLVSKLDSGVPDRFSGSGSGTDFTLKISRVEAEDVGVYFCWQGTHLPQTFGGGTKVEIK

SEQ ID NO: 32 - DNA, 336 bp, Artificial Sequence
  Nucleic acid sequence of light chain
gacgtggtcatgacacagagcccactgtctctgcctgtgaccctgggacagccagcctctatctcctgcaagtccagccagtccctgctgcacagcgtgggcaagacatacctgaactggctgcagcagaggccaggacagagcccaaggcggctgatctatctggtgtctaagctggactccggcgtgcctgatagattcagcggctctggctccggcaccgactttacactgaagatctctcgcgtggaggctgaggatgtgggcgtgtacttctgttggcagggcacccatctgccacagacatttggcggcggcaccaaggtggagatcaag

SEQ ID NO: 33 - protein, 123 aa, Artificial Sequence
  43E5-01 Amino acid sequence of the heavy chain
QVQLVQSGAEVKKPGASVKVSCKASGYTFTDYEMHWVRQAPGQGLEWMGAIDPETGGTAYNQKFKGRVTMTADKSISTAYMELSRLRSDDTAVYYCRRGANLNHYGNDEGSYWGQGTLVTVSS

SEQ ID NO: 34 - DNA, 369 bp, Artificial Sequence
  43E5-01 Nucleic acid sequence of the heavy chain
caggtgcagctggtgcagtccggagctgaggtgaagaagccaggagcctccgtgaaggtgtcttgcaaggcctccggctacaccttcacagactatgagatgcactgggtgaggcaggctccaggacagggactggagtggatgggagctatcgatcctgagaccggaggaacagcttacaaccagaagtttaagggcagagtgaccatgacagccgacaagtctatctccaccgcttatatggagctgagcagactgcgctctgacgatacagccgtgtactattgtaggcggggcgctaacctgaatcattacggcaatgatgagggctcctattggggccagggcaccctggtgacagtgtccagc

SEQ ID NO: 35 - protein, 123 aa, Artificial Sequence
  43E5-02 Amino acid sequence of the heavy chain
QVQLVQSGAEVKKPGASVKVSCKASGYTFTDYEMHWVRQAPGQGLEWIGAIDPETGGTAYNQKFKGRATLTADKSISTAYMELSRLRSDDTAVYYCRRGANLNHYGNDEGSYWGQGTLVTVSS

SEQ ID NO: 36 - DNA, 369 bp, Artificial Sequence
  43E5-02 Nucleic acid sequence of the heavy chain
caggtgcagctggtgcagtccggagctgaggtgaagaagccaggagcctccgtgaaggtgtcttgcaaggcctccggctacaccttcacagactatgagatgcactgggtgaggcaggctccaggacagggactggagtggatcggagctatcgatcctgagaccggaggaacagcttacaaccagaagtttaagggcagagccaccctgacagctgacaagtctatctccaccgcctatatggagctgagcagactgcgctctgacgatacagccgtgtactattgtaggcggggcgctaacctgaatcattacggcaatgatgagggctcctattggggccagggcaccctggtgacagtgtccagc

SEQ ID NO: 37 - protein, 123 aa, Artificial Sequence
  43E5-05 Amino acid sequence of the heavy chain
QVQLVQSGAEVKKPGSSVKVSCKASGYTFTDYEMHWVRQAPGQGLEWMGAIDPETGGTAYNQKFKGRVTITADKSTSTAYMELSSLRSEDTAVYYCRRGANLNHYGNDEGSYWGQGTLVTVSS

SEQ ID NO: 38 - DNA, 369 bp, Artificial Sequence
  43E5-05 Nucleic acid sequence of the heavy chain
caggtgcagctggtgcagtccggagctgaggtgaagaagccaggctccagcgtgaaggtgtcttgcaaggcttccggctacaccttcacagactatgagatgcactgggtgaggcaggctccaggacagggactggagtggatgggagctatcgatcctgagaccggaggaacagcttacaaccagaagtttaagggcagagtgaccatcacagccgacaagtccaccagcacagcttatatggagctgtcttccctgcgcagcgaggataccgccgtgtactattgtaggcggggcgctaacctgaatcattacggcaatgacgagggctcttattggggccagggcaccctggtgacagtgagctct

SEQ ID NO: 39 - protein, 123 aa, Artificial Sequence
  43E5-06 Amino acid sequence of the heavy chain
QVQLVQSGAEVKKPGSSVKVSCKASGYTFTDYEMHWVRQAPGQGLEWIGAIDPETGGTAYNQKFKGRATLTADKSTSTAYMELSSLRSEDTAVYYCRRGANLNHYGNDEGSYWGQGTLVTVSS

SEQ ID NO: 40 - DNA, 369 bp, Artificial Sequence
  43E5-06 Nucleic acid sequence of the heavy chain
caggtgcagctggtgcagtccggagctgaggtgaagaagccaggctccagcgtgaaggtgtcttgcaaggcttccggctacaccttcacagactatgagatgcactgggtgaggcaggctccaggacagggactggagtggatcggagctatcgatcctgagaccggaggaacagcttacaaccagaagtttaagggcagagccaccctgacagctgacaagtccaccagcacagcttatatggagctgtcttccctgcgcagcgaggataccgccgtgtactattgtaggcggggcgctaacctgaatcattacggcaatgacgagggctcttattggggccagggcaccctggtgacagtgagctct

SEQ ID NO: 41 - protein, 107 aa, Artificial Sequence
  Amino acid sequence of the light chain
DIQMTQSPSSLSASVGDRVTITCRASQDISNYLNWYQQKPGKAPKLLIYYTSRLHSGVPSRFSGSGSGTDYTLTISSLQPEDFATYFCQQGNTLPRTFGGGTKVEIK

SEQ ID NO: 42 - DNA, 321 bp, Artificial Sequence
  Nucleic acid sequence of the light chain
gacatccagatgacccagagccccagcagcctgagcgccagcgtgggcgacagagtgaccatcacctgcagagccagccaggacatcagcaactacctgaactggtaccagcagaagcccggcaaggcccccaagctgctgatctactacaccagcagactgcacagcggcgtgcccagcagattcagcggcagcggcagcggcaccgactacaccctgaccatcagcagcctgcagcccgaggacttcgccacctacttctgccagcagggcaacaccctgcccagaaccttcggcggcggcaccaaggtggagatcaag

SEQ ID NO: 43 - protein, 121 aa, Artificial Sequence
  138E12-01 Amino acid sequence of the heavy chain
QVQLQESGPGLVKPSETLSLTCTVSGFSLTGYGVNWIRQPPGKGLEWIGMIWFDGSTDYNSALKSRVTISKDNSKSQVSLKLSSVTAADTAVYYCAREGYYYGTTYYFDYWGQGTTVTVSS

SEQ ID NO: 44 - DNA, 363 bp, Artificial Sequence
  138E12-01 Nucleic acid sequence of the heavy chain
caggtgcagctgcaggagagcggccccggcctggtgaagcccagcgagaccctgagcctgacctgcaccgtgagcggcttcagcctgaccggctacggcgtgaactggatcagacagccccccggcaagggcctggagtggatcggcatgatctggttcgacggcagcaccgactacaacagcgccctgaagagcagagtgaccatcagcaaggacaacagcaagagccaggtgagcctgaagctgagcagcgtgaccgccgccgacaccgccgtgtactactgcgccagagagggctactactacggcaccacctactacttcgactactggggccagggcaccaccgtgaccgtgagcagc

SEQ ID NO: 45 - protein, 121 aa, Artificial Sequence
  138E12-02 Amino acid sequence of the heavy chain
QVQLQESGPGLVKPSETLSLTCTVSGFSLTGYGVNWIRQPPGKGLEWLGMIWFDGSTDYNSALKSRLTISKDNSKSQVSLKLSSVTAADTAVYYCAREGYYYGTTYYFDYWGQGTTVTVSS

SEQ ID NO: 46 - DNA, 363 bp, Artificial Sequence
  138E12-02 Nucleic acid sequence of the heavy chain
caggtgcagctgcaggagagcggccccggcctggtgaagcccagcgagaccctgagcctgacctgcaccgtgagcggcttcagcctgaccggctacggcgtgaactggatcagacagccccccggcaagggcctggagtggctgggcatgatctggttcgacggcagcaccgactacaacagcgccctgaagagcagactgaccatcagcaaggacaacagcaagagccaggtgagcctgaagctgagcagcgtgaccgccgccgacaccgccgtgtactactgcgccagagagggctactactacggcaccacctactacttcgactactggggccagggcaccaccgtgaccgtgagcagc

SEQ ID NO: 47 - protein, 121 aa, Artificial Sequence
  138E12-03 Amino acid sequence of the heavy chain
QVQLQESGPGLVKPSETLSLTCTVSGFSLTGYGVNWIRQPPGKGLEWLGMIWFEGSTDYNSALKSRLTISKDNSKSQVSLKLSSVTAADTAVYYCAREGYYYGTTYYFDYWGQGTTVTVSS

SEQ ID NO: 48 - DNA, 363 bp, Artificial Sequence
  138E12-03 Nucleic acid sequence of the heavy chain
caggtgcagctgcaggagagcggccccggcctggtgaagcccagcgagaccctgagcctgacctgcaccgtgagcggcttcagcctgaccggctacggcgtgaactggatcagacagccccccggcaagggcctggagtggctgggcatgatctggttcgagggcagcaccgactacaacagcgccctgaagagcagactgaccatcagcaaggacaacagcaagagccaggtgagcctgaagctgagcagcgtgaccgccgccgacaccgccgtgtactactgcgccagagagggctactactacggcaccacctactacttcgactactggggccagggcaccaccgtgaccgtgagcagc

SEQ ID NO: 49 - protein, 121 aa, Artificial Sequence
  138E12-04 Amino acid sequence of the heavy chain
QVQLQESGPGLVKPSETLSLTCTVSGFSLTGYGVNWIRQPPGKGLEWLGMIWFDASTDYNSALKSRLTISKDNSKSQVSLKLSSVTAADTAVYYCAREGYYYGTTYYFDYWGQGTTVTVSS

SEQ ID NO: 50 - DNA, 363 bp, Artificial Sequence
  138E12-04 Nucleic acid sequence of the heavy chain
caggtgcagctgcaggagagcggccccggcctggtgaagcccagcgagaccctgagcctgacctgcaccgtgagcggcttcagcctgaccggctacggcgtgaactggatcagacagccccccggcaagggcctggagtggctgggcatgatctggttcgacgccagcaccgactacaacagcgccctgaagagcagactgaccatcagcaaggacaacagcaagagccaggtgagcctgaagctgagcagcgtgaccgccgccgacaccgccgtgtactactgcgccagagagggctactactacggcaccacctactacttcgactactggggccagggcaccaccgtgaccgtgagcagc

SEQ ID NO: 51 - protein, 121 aa, Artificial Sequence
  138E12-05 Amino acid sequence of the heavy chain
QVQLQESGPGLVKPSETLSLTCTVSGFSLTGYGVNWIRQPPGKGLEWLGMIWFDGSTDYQSALKSRLTISKDNSKSQVSLKLSSVTAADTAVYYCAREGYYYGTTYYFDYWGQGTTVTVSS

SEQ ID NO: 52 - DNA, 363 bp, Artificial Sequence
  138E12-05 Nucleic acid sequence of the heavy chain
caggtgcagctgcaggagagcggccccggcctggtgaagcccagcgagaccctgagcctgacctgcaccgtgagcggcttcagcctgaccggctacggcgtgaactggatcagacagccccccggcaagggcctggagtggctgggcatgatctggttcgacggcagcaccgactaccagagcgccctgaagagcagactgaccatcagcaaggacaacagcaagagccaggtgagcctgaagctgagcagcgtgaccgccgccgacaccgccgtgtactactgcgccagagagggctactactacggcaccacctactacttcgactactggggccagggcaccaccgtgaccgtgagcagc

SEQ ID NO: 53 - protein, 121 aa, Artificial Sequence
  138E12-06 Amino acid sequence of the heavy chain
QVQLQESGPGLVKPSETLSLTCTVSGFSLTGYGVNWIRQPPGKGLEWLGMIWFDGSTDYNTALKSRLTISKDNSKSQVSLKLSSVTAADTAVYYCAREGYYYGTTYYFDYWGQGTTVTVSS

SEQ ID NO: 54 - DNA, 363 bp, Artificial Sequence
  138E12-06 Nucleic acid sequence of the heavy chain
caggtgcagctgcaggagagcggccccggcctggtgaagcccagcgagaccctgagcctgacctgcaccgtgagcggcttcagcctgaccggctacggcgtgaactggatcagacagccccccggcaagggcctggagtggctgggcatgatctggttcgacggcagcaccgactacaacaccgccctgaagagcagactgaccatcagcaaggacaacagcaagagccaggtgagcctgaagctgagcagcgtgaccgccgccgacaccgccgtgtactactgcgccagagagggctactactacggcaccacctactacttcgactactggggccagggcaccaccgtgaccgtgagcagc

SEQ ID NO: 55 - protein, 121 aa, Artificial Sequence
  138E12-07 Amino acid sequence of the heavy chain
QVQLQESGPGLVKPSETLSLTCTVSGFSLTGYGVNWIRQPPGKGLEWIGMIWFEGSTDYQSALKSRVTISVDTSKNQFSLKLSSVTAADTAVYYCAREGYYYGTTYYFDYWGQGTTVTVSS

SEQ ID NO: 56 - DNA, 363 bp, Artificial Sequence
  138E12-07 Nucleic acid sequence of the heavy chain
caggtgcagctgcaggagagcggccccggcctggtgaagcccagcgagaccctgagcctgacctgcaccgtgagcggcttcagcctgaccggctacggcgtgaactggatcagacagccccccggcaagggcctggagtggatcggcatgatctggttcgagggcagcaccgactaccagagcgccctgaagagcagagtgaccatcagcgtggacaccagcaagaaccagttcagcctgaagctgagcagcgtgaccgccgccgacaccgccgtgtactactgcgccagagagggctactactacggcaccacctactacttcgactactggggccagggcaccaccgtgaccgtgagcagc

SEQ ID NO: 57 - protein, 121 aa, Artificial Sequence
  138E12-08 Amino acid sequence of the heavy chain
QVQLQESGPGLVKPSETLSLTCTVSGFSLTGYGVNWIRQPPGKGLEWIGMIWFEGSTDYNSALKSRVTISKDNSKSQVSLKLSSVTAADTAVYYCAREGYYYGTTYYFDYWGQGTTVTVSS

SEQ ID NO: 58 - DNA, 363 bp, Artificial Sequence
  138E12-08 Nucleic acid sequence of the heavy chain
caggtgcagctgcaggagagcggccccggcctggtgaagcccagcgagaccctgagcctgacctgcaccgtgagcggcttcagcctgaccggctacggcgtgaactggatcagacagccccccggcaagggcctggagtggatcggcatgatctggttcgagggcagcaccgactacaacagcgccctgaagagcagagtgaccatcagcaaggacaacagcaagagccaggtgagcctgaagctgagcagcgtgaccgccgccgacaccgccgtgtactactgcgccagagagggctactactacggcaccacctactacttcgactactggggccagggcaccaccgtgaccgtgagcagc

SEQ ID NO: 59 - protein, 121 aa, Artificial Sequence
  138E12-09 Amino acid sequence of the heavy chain
QVQLQESGPGLVKPSETLSLTCTVSGFSLTGYGVNWIRQPPGKGLEWIGMIWFDGSTDYQSALKSRVTISKDNSKSQVSLKLSSVTAADTAVYYCAREGYYYGTTYYFDYWGQGTTVTVSS

SEQ ID NO: 60 - DNA, 363 bp, Artificial Sequence
  138E12-09 Nucleic acid sequence of the heavy chain
caggtgcagctgcaggagagcggccccggcctggtgaagcccagcgagaccctgagcctgacctgcaccgtgagcggcttcagcctgaccggctacggcgtgaactggatcagacagccccccggcaagggcctggagtggatcggcatgatctggttcgacggcagcaccgactaccagagcgccctgaagagcagagtgaccatcagcaaggacaacagcaagagccaggtgagcctgaagctgagcagcgtgaccgccgccgacaccgccgtgtactactgcgccagagagggctactactacggcaccacctactacttcgactactggggccagggcaccaccgtgaccgtgagcagc

SEQ ID NO: 61 - protein, 121 aa, Artificial Sequence
  138E12-10 Amino acid sequence of the heavy chain
QVQLQESGPGLVKPSETLSLTCTVSGFSLTGYGVNWIRQPPGKGLEWIGMIWFEGSTDYQSALKSRVTISKDNSKSQVSLKLSSVTAADTAVYYCAREGYYYGTTYYFDYWGQGTTVTVSS

SEQ ID NO: 62 - DNA, 363 bp, Artificial Sequence
  138E12-10 Nucleic acid sequence of the heavy chain
caggtgcagctgcaggagagcggccccggcctggtgaagcccagcgagaccctgagcctgacctgcaccgtgagcggcttcagcctgaccggctacggcgtgaactggatcagacagccccccggcaagggcctggagtggatcggcatgatctggttcgagggcagcaccgactaccagagcgccctgaagagcagagtgaccatcagcaaggacaacagcaagagccaggtgagcctgaagctgagcagcgtgaccgccgccgacaccgccgtgtactactgcgccagagagggctactactacggcaccacctactacttcgactactggggccagggcaccaccgtgaccgtgagcagc

SEQ ID NO: 63 - protein, 121 aa, Artificial Sequence
  138E12-11 Amino acid sequence of the heavy chain
QVQLQESGPGLVKPSETLSLTCTVSGFSLTGYGVNWIRQPPGKGLEWLGMIWFEGSTDYQSALKSRLTISKDNSKSQVSLKLSSVTAADTAVYYCAREGYYYGTTYYFDYWGQGTTVTVSS

SEQ ID NO: 64 - DNA, 363 bp, Artificial Sequence
  138E12-11 Nucleic acid sequence of the heavy chain
caggtgcagctgcaggagagcggccccggcctggtgaagcccagcgagaccctgagcctgacctgcaccgtgagcggcttcagcctgaccggctacggcgtgaactggatcagacagccccccggcaagggcctggagtggctgggcatgatctggttcgagggcagcaccgactaccagagcgccctgaagagcagactgaccatcagcaaggacaacagcaagagccaggtgagcctgaagctgagcagcgtgaccgccgccgacaccgccgtgtactactgcgccagagagggctactactacggcaccacctactacttcgactactggggccagggcaccaccgtgaccgtgagcagc